European Patent Application EP 4 722 358 A1, published April 8, 2026. Title: Glycerol dehydratase variants. Applicant: AJOU UNIVERSITY INDUSTRY-ACADEMIC COOPERATION FOUNDATION. The sequence listing filed with the application follows.

SEQUENCE LISTING (24 sequences)

SEQ ID NO: 1 - protein, 555 aa, Klebsiella pneumoniae
MKRSKRFAVLAQRPVNQDGLIGEWPEEGLIAMDSPFDPVSSVKVDNGLIVELDGKRRDQFDMIDRFIADYAINVERTEQAMRLEAVEIARMLVDIHVSREEIIAITTAITPAKAVEVMAQMNVVEMMMALQKMRARRTPSNQCHVTNLKDNPVQIAADAAEAGIRGFSEQETTVGIARYAPFNALALLVGSQCGRPGVLTQCSVEEATELELGMRGLTSYAETVSVYGTEAVFTDGDDTPWSKAFLASAYASRGLKMRYTSGTGSEALMGYSESKSMLYLESRCIFITKGAGVQGLQNGAVSCIGMTGAVPSGIRAVLAENLIASMLDLEVASANDQTFSHSDIRRTARTLMQMLPGTDFIFSGYSAVPNYDNMFAGSNFDAEDFDDYNILQRDLMVDGGLRPVTEAETIAIRQKAARAIQAVFRELGLPPIADEEVEAATYAHGSNEMPPRNVVEDLSAVEEMMKRNITGLDIVGALSRSGFEDIASNILNMLRQRVTGDYLQTSAILDRQFEVVSAVNDINDYQGPGTGYRISAERWAEIKNIPGVVQPDTIE

SEQ ID NO: 2 - protein, 194 aa, Klebsiella pneumoniae
MQQTTQIQPSFTLKTREGGVASADERADEVVIGVGPAFDKHQHHTLIDMPHGAILKELIAGVEEEGLHARVVRILRTSDVSFMAWDAANLSGSGIGIGIQSKGTTVIHQRDLLPLSNLELFSQAPLLTLETYRQIGKNAARYARKESPSPVPVVNDQMVRPKFMAKAALFHIKETKHVVQDAEPVTLHIDLVRE

SEQ ID NO: 3 - protein, 141 aa, Klebsiella pneumoniae
MSEKTMRVQDYPLATRCPEHILTPTGKPLTDITLEKVLSGEVGPQDVRISRQTLEYQAQIAEQMQRHAVARNFRRAAELIAIPDERILAIYNALRPFRSSQAELLAIADELEHTWHATVNAAFVRESAEVYQQRHKLRKGS

SEQ ID NO: 4 - protein, 754 aa, synthetic construct
MKRSKRFAVLAQRPVNQDGLIGEWPEEGLIAMDSPFDPVSSVKVDNGLIVELDGKRRDQFDMIDRFIADYAINVERTEQAMRLEAVEIARMLVDIHVSREEIIAITTAITPAKAVEVMAQMNVVEMMMALQKMRARRTPSNQCHVTNLKDNPVQIAADAAEAGIRGFSEQETTVGIARYAPFNALALLVGSQCGRPGVLTQCSVEEATELELGMRGLTSYAETVSVYGTEAVFTDGDDTPWSKAFLASAYASRGLKMRYTSGTGSEALMGYSESKSMLYLESRCIFITKGAGVQGLQNGAVSCIGMTGAVPSGIRAVLAENLIASMLDLEVASANDQTFSHSDIRRTARTLMQMLPGTDFIFSGYSAVPNYDNMFAGSNFDAEDFDDYNILQRDLMVDGGLRPVTEAETIAIRQKAARAIQAVFRELGLPPIADEEVEAATYAHGSNEMPPRNVVEDLSAVEEMMKRNITGLDIVGALSRSGFEDIASNILNMLRQRVTGDYLQTSAILDRQFEVVSAVNDINDYQGPGTGYRISAERWAEIKNIPGVVQPDTIEQGGIPVQQTTQIQPSFTLKTREGGVASADERADEVVIGVGPAFDKHQHHTLIDMPHGAILKELIAGVEEEGLHARVVRILRTSDVSFMAWDAANLSGSGIGIGIQSKGTTVIHQRDLLPLSNLELFSQAPLLTLETYRQIGKNAARYARKESPSPVPVVNDQMVRPKFMAKAALFHIKETKHVVQDAEPVTLHIDLVRE

SEQ ID NO: 5 - protein, 754 aa, synthetic construct
MKRSKRFAVLAQRPVNQDGLIGEWPEEGLIAMDSPFDPVSSVKVDNGLIVELDGKRRDQFDMIDRFIADYAINVERTEQAMRLEAVEIARMLVDIHVSREEIIAITTAITPAKAVEVMAQMNVVEMMMALQKMRARRTPSNQCHVTNLKDNPVQIAADAAEAGIRGFSEQETTVGIMRYAPFNALALLVGSQCGRPGVLTQCSVEEATELELGMRGLTSYAETVSVYGTEAVFTDGDDTPWSKAFLASAYASRGLKMRYTSGTGSEALMGYSESKSMLYLESRCIFITKGAGVQGLQNGAVSCIGMTGAVPSGIRAVLAENLIASMLDLEVASANDQTFSHSDIRRTARTLMQMLPGTDFIFSGYSAVPNYDNMFAGSNFDAEDFDDYNILQRDLMVDGGLRPVTEAETIAIRQKAARAIQAVFRELGLPPIADEEVEAATYAHGSNEMPPRNVVEDLSAVEEMMKRNITGLDIVGALSRSGFEDIASNILNMLRQRVTGDYLQTSAILDRQFEVVSAVNDINDYQGPGTGYRISAERWAEIKNIPGVVQPDTIEQGGIPVQQTTQIQPSFTLKTREGGVASADERADEVVIGVGPAFDKHQHHTLIDMPHGAILKELIAGVEEEGLHARVVRILRTSDVSFMAWDAANLSGSGIGIGIQSKGTTVIHQRDLLPLSNLELFSQAPLLTLETYRQIGKNAARYARKESPSPVPVVNDQMVRPKFMAKAALFHIKETKHVVQDAEPVTLHIDLVRE

SEQ ID NO: 6 - protein, 754 aa, synthetic construct
MKRSKRFAVLAQRPVNQDGLIGEWPEEGLIAMDSPFDPVSSVKVDNGLIVELDGKRRDQFDMIDRFIADYAINVERTEQAMRLEAVEIARMLVDIHVSREEIIAITTAITPAKAVEVMAQMNVVEMMMALQKMRARRTPSNQCHVTNLKDNPVQIAADAAEAGIRGFSEQETTVGIARYAPFNALALLVGSQCGRPGVLTQCSVEEATELELGMRGLTSYAETVSVYGTEAVFTDGDDTPWSKAFLASAYASRGLKMRYTSGTGSEALMGYSESKSMLYLESRCIFITKGAGVQGLQNGAVSCIGMTGAVPSGIRAVLAENLIASMLDLEVASANDQTFSHSDIRRTARTLMQMLPGTDFIFSGYSAVPNYDNMFAGSNFDAEDFDDYNILQRDLMVDGGLRPVTEAETIAIRQKAARAIQAVFRELGLPPIADEEVEAATYAHGSNEMPPRNVWEDLSAVEEMMKRNITGLDIVGALSRSGFEDIASNILNMLRQRVTGDYLQTSAILDRQFEVVSAVNDINDYQGPGTGYRISAERWAEIKNIPGVVQPDTIEQGGIPVQQTTQIQPSFTLKTREGGVASADERADEVVIGVGPAFDKHQHHTLIDMPHGAILKELIAGVEEEGLHARVVRILRTSDVSFMAWDAANLSGSGIGIGIQSKGTTVIHQRDLLPLSNLELFSQAPLLTLETYRQIGKNAARYARKESPSPVPVVNDQMVRPKFMAKAALFHIKETKHVVQDAEPVTLHIDLVRE

SEQ ID NO: 7 - protein, 754 aa, synthetic construct
MKRSKRFAVLAQRPVNQDGLIGEWPEEGLIAMDSPFDPVSSVKVDNGLIVELDGKRRDQFDMIDRFIADYAINVERTEQAMRLEAVEIARMLVDIHVSREEIIAITTAITPAKAVEVMAQMNVVEMMMALQKMRARRTPSNQCHVTNLKDNPVQIAADAAEAGIRGFSEQETTVGIARYAPFNALALLVGSQCGRPGVLTQCSVEEATELELGMRGLTSYAETVSVYGTEAVFTDGDDTPWSKAFLASAYASRGLKMRYTSGTGSEALMGYSESKSMLYLESRCIFITKGAGVQGLQNGAVSCIGMTGAVPSGIRAVLAENLIASMLDLEVASANDQTFSHSDIRRTARTLMQMLPGTDFIFSGYSAVPNYDNMFAGSNFDAEDFDDYNILQRDLMVDGGLRPVTEAETIAIRQKAARAIQAVFRELGLPPIADEEVEAATYAHGSNEMPPRNVVEDLSAVEEMMKRNITGLDIVGALSRSGFEDIASNILNMLRQRVTGDYLQTSAILDRQFEVVSAVNDINDYQGPGTGYRISAERWAEIKNIPGVVQPDTIEQGGIPVQQTTQIQPSFTLKTREGGVASADERADEVVIGVGPAFDKHQHHTLIDMPHGAILKELIAGVEEEGLHARVVRILRTSDVSFMAWDAANLSGSGIGIGIQSKGTTVIHQRDLWPLSNLELFSQAPLLTLETYRQIGKNAARYARKESPSPVPVVNDQMVRPKFMAKAALFHIKETKHVVQDAEPVTLHIDLVRE

SEQ ID NO: 8 - protein, 754 aa, synthetic construct
MKRSKRFAVLAQRPVNQDGLIGEWPEEGLIAMDSPFDPVSSVKVDNGLIVELDGKRRDQFDMIDRFIADYAINVERTEQAMRLEAVEIARMLVDIHVSREEIIAITTAITPAKAVEVMAQMNVVEMMMALQKMRARRTPSNQCHVTNLKDNPVQIAADAAEAGIRGFSEQETTVGIARYAPFNALALLVGSQCGRPGVLTQCSVEEATELELGMRGLTSYAETVSVYGTEAVFTDGDDTPWSKAFLASAYASRGLKMRYTSGTGSEALMGYSESKSMLYLESRCIFITKGAGVQGLQNGAVSCIGMTGAVPSGIRAVLAENLIASMLDLEVASANDQTFSHSDIRRTARTLMQMLPGTDFIFSGYSAVPNYDNMFAGSNFDAEDFDDYNILQRDLMVDGGLRPVTEAETIAIRQKAARAIQAVFRELGLPPIADEEVEAATYAHGSNEMPPRNVVEDLSAVEEMMKRNITGLDIVGALSRSGFEDIASNILNMLRQRVTGDYLQTSAILDRQFEVVSAVNDINDYQGPGTGYRISAERWAEIKNIPGVVQPDTIEQGGIPVQQTTQIQPSFTLKTREGGVASADERADEVVIGVGPAFDKHQHHTLIDMPHGAILKELIAGVEEEGLHARVVRILRTSDVSFMAWDAANLSGSGIGIGIQSKGTTVIHQRDLFPLSNLELFSQAPLLTLETYRQIGKNAARYARKESPSPVPVVNDQMVRPKFMAKAALFHIKETKHVVQDAEPVTLHIDLVRE

SEQ ID NO: 9 - protein, 754 aa, synthetic construct
MKRSKRFAVLAQRPVNQDGLIGEWPEEGLIAMDSPFDPVSSVKVDNGLIVELDGKRRDQFDMIDRFIADYAINVERTEQAMRLEAVEIARMLVDIHVSREEIIAITTAITPAKAVEVMAQMNVVEMMMALQKMRARRTPSNQCHVTNLKDNPVQIAADAAEAGIRGFSEQETTVGIARYAPFNALALLVGSQCGRPGVLTQCSVEEATELELGMRGLTSYAETVSVYGTEAVFTDGDDTPWSKAFLASAYASRGLKMRYTSGTGSEALMGYSESKSMLYLESRCIFITKGAGVQGLQNGAVSCIGMTGAVPSGIRAVLAENLIASMLDLEVASANDQTFSHSDIRRTARTLMQMLPGTDFIFSGYSAVPNYDNMFAGSNFDAEDFDDYNILQRDLMVDGGLRPVTEAETIAIRQKAARAIQAVFRELGLPPIADEEVEAATYAHGSNEMPPRNVVEDLSAVEEMMKRNITGLDIVGALSRSGFEDIASNILNMLRQRVTGDYLQTSAILDRQFEVVSAVNDINDYQGPGTGYRISAERWAEIKNIPGVVQPDTIEQGGIPVQQTTQIQPSFTLKTREGGVASADERADEVVIGVGPAFDKHQHHTLIDMPHGAILKELIAGVEEEGLHARVVRILRTSDVSFMAWDAANLSGSGIGIGIQSKGTTVIHQRDLLPLSNLELFSQAPLLTLETYRQIGKNAARYARKESPSPVPVVNDQWVRPKFMAKAALFHIKETKHVVQDAEPVTLHIDLVRE

SEQ ID NO: 10 - protein, 754 aa, synthetic construct
MKRSKRFAVLAQRPVNQDGLIGEWPEEGLIAMDSPFDPVSSVKVDNGLIVELDGKRRDQFDMIDRFIADYAINVERTEQAMRLEAVEIARMLVDIHVSREEIIAITTAITPAKAVEVMAQMNVVEMMMALQKMRARRTPSNQCHVTNLKDNPVQIAADAAEAGIRGFSEQETTVGIMRYAPFNALALLVGSQCGRPGVLTQCSVEEATELELGMRGLTSYAETVSVYGTEAVFTDGDDTPWSKAFLASAYASRGLKMRYTSGTGSEALMGYSESKSMLYLESRCIFITKGAGVQGLQNGAVSCIGMTGAVPSGIRAVLAENLIASMLDLEVASANDQTFSHSDIRRTARTLMQMLPGTDFIFSGYSAVPNYDNMFAGSNFDAEDFDDYNILQRDLMVDGGLRPVTEAETIAIRQKAARAIQAVFRELGLPPIADEEVEAATYAHGSNEMPPRNVVEDLSAVEEMMKRNITGLDIVGALSRSGFEDIASNILNMLRQRVTGDYLQTSAILDRQFEVVSAVNDINDYQGPGTGYRISAERWAEIKNIPGVVQPDTIEQGGIPVQQTTQIQPSFTLKTREGGVASADERADEVVIGVGPAFDKHQHHTLIDMPHGAILKELIAGVEEEGLHARVVRILRTSDVSFMAWDAANLSGSGIGIGIQSKGTTVIHQRDLWPLSNLELFSQAPLLTLETYRQIGKNAARYARKESPSPVPVVNDQMVRPKFMAKAALFHIKETKHVVQDAEPVTLHIDLVRE

SEQ ID NO: 11 - protein, 754 aa, synthetic construct
MKRSKRFAVLAQRPVNQDGLIGEWPEEGLIAMDSPFDPVSSVKVDNGLIVELDGKRRDQFDMIDRFIADYAINVERTEQAMRLEAVEIARMLVDIHVSREEIIAITTAITPAKAVEVMAQMNVVEMMMALQKMRARRTPSNQCHVTNLKDNPVQIAADAAEAGIRGFSEQETTVGIMRYAPFNALALLVGSQCGRPGVLTQCSVEEATELELGMRGLTSYAETVSVYGTEAVFTDGDDTPWSKAFLASAYASRGLKMRYTSGTGSEALMGYSESKSMLYLESRCIFITKGAGVQGLQNGAVSCIGMTGAVPSGIRAVLAENLIASMLDLEVASANDQTFSHSDIRRTARTLMQMLPGTDFIFSGYSAVPNYDNMFAGSNFDAEDFDDYNILQRDLMVDGGLRPVTEAETIAIRQKAARAIQAVFRELGLPPIADEEVEAATYAHGSNEMPPRNVVEDLSAVEEMMKRNITGLDIVGALSRSGFEDIASNILNMLRQRVTGDYLQTSAILDRQFEVVSAVNDINDYQGPGTGYRISAERWAEIKNIPGVVQPDTIEQGGIPVQQTTQIQPSFTLKTREGGVASADERADEVVIGVGPAFDKHQHHTLIDMPHGAILKELIAGVEEEGLHARVVRILRTSDVSFMAWDAANLSGSGIGIGIQSKGTTVIHQRDLLPLSNLELFSQAPLLTLETYRQIGKNAARYARKESPSPVPVVNDQWVRPKFMAKAALFHIKETKHVVQDAEPVTLHIDLVRE

SEQ ID NO: 12 - protein, 754 aa, synthetic construct
MKRSKRFAVLAQRPVNQDGLIGEWPEEGLIAMDSPFDPVSSVKVDNGLIVELDGKRRDQFDMIDRFIADYAINVERTEQAMRLEAVEIARMLVDIHVSREEIIAITTAITPAKAVEVMAQMNVVEMMMALQKMRARRTPSNQCHVTNLKDNPVQIAADAAEAGIRGFSEQETTVGIMRYAPFNALALLVGSQCGRPGVLTQCSVEEATELELGMRGLTSYAETVSVYGTEAVFTDGDDTPWSKAFLASAYASRGLKMRYTSGTGSEALMGYSESKSMLYLESRCIFITKGAGVQGLQNGAVSCIGMTGAVPSGIRAVLAENLIASMLDLEVASANDQTFSHSDIRRTARTLMQMLPGTDFIFSGYSAVPNYDNMFAGSNFDAEDFDDYNILQRDLMVDGGLRPVTEAETIAIRQKAARAIQAVFRELGLPPIADEEVEAATYAHGSNEMPPRNVVEDLSAVEEMMKRNITGLDIVGALSRSGFEDIASNILNMLRQRVTGDYLQTSAILDRQFEVVSAVNDINDYQGPGTGYRISAERWAEIKNIPGVVQPDTIEQGGIPVQQTTQIQPSFTLKTREGGVASADERADEVVIGVGPAFDKHQHHTLIDMPHGAILKELIAGVEEEGLHARVVRILRTSDVSFMAWDAANLSGSGIGIGIQSKGTTVIHQRDLWPLSNLELFSQAPLLTLETYRQIGKNAARYARKESPSPVPVVNDQWVRPKFMAKAALFHIKETKHVVQDAEPVTLHIDLVRE

SEQ ID NO: 13 - DNA, 1668 bp, Klebsiella pneumoniae
  source 1..1668: mol_type = genomic DNA
atgaaaagatcaaaacgatttgcagtactggcccagcgccccgtcaatcaggacgggctgattggcgagtggcctgaagaggggctgatcgccatggacagcccctttgacccggtctcttcagtaaaagtggacaacggtctgatcgtcgagctggacggcaaacgccgggaccagtttgacatgatcgaccgatttatcgccgattacgcgatcaacgttgagcgcacagagcaggcaatgcgcctggaggcggtggaaatagcccgcatgctggtggatattcacgtcagtcgggaggagatcattgccatcactaccgccatcacgccggccaaagcggtcgaggtgatggcgcagatgaacgtggtggagatgatgatggcgctgcagaagatgcgtgcccgccggaccccctccaaccagtgccacgtcaccaatctcaaagataatccggtgcagattgctgctgacgccgccgaggccgggatccgcggcttctcagaacaggagaccacggtcggtatcgcgcgctatgcgccgtttaacgccctggcgctgttggtcggttcgcagtgcggccgccccggcgttttgacgcagtgctcggtggaagaggccaccgagctggagctgggcatgcgtggcttaaccagctacgccgagacggtgtcggtctacggcaccgaagcggtatttaccgacggcgatgatactccgtggtcaaaggcgttcctcgcctcggcctacgcctcccgcgggttgaaaatgcgctacacctccggcaccggatccgaagcgctgatgggctattcggagagcaagtcgatgctctacctcgaatcgcgctgcatcttcattaccaaaggcgccggggttcaggggctgcaaaacggcgcggtgagctgtatcggcatgaccggcgctgtgccgtcgggcattcgggcggtgctggcggaaaacctgatcgcctctatgctcgacctcgaagtggcgtccgccaacgaccagactttctcccactcggatattcgccgcaccgcgcgcaccctgatgcagatgctgccgggcaccgactttattttctccggctacagcgcggtgccgaactacgacaacatgttcgccggctcgaacttcgatgcggaagattttgatgattacaacatcctgcagcgtgacctgatggttgacggcggcctgcgtccggtgaccgaggcggaaaccattgccattcgccagaaagcggcgcgggcgatccaggcggttttccgcgagctggggctgccgccaatcgccgacgaggaggtggaggccgccacctacgcgcacggtagcaacgagatgccgccgcgtaacgtggtggaggatctgagtgcggtggaagagatgatgaagcgcaacatcaccggcctcgatattgtcggcgcgctgagccgcagcggctttgaggatatcgccagcaatattctcaatatgctgcgccagcgggtcaccggcgattacctgcagacctcggccattctcgatcggcagttcgaggtggtgagtgcggtcaacgacatcaatgactatcaggggccgggcaccggctatcgcatctctgccgaacgctgggcggagatcaaaaatattccgggcgtggttcagcccgacaccattgaataa

SEQ ID NO: 14 - DNA, 585 bp, Klebsiella pneumoniae
  source 1..585: mol_type = genomic DNA
gtgcaacagacaacccaaattcagccctcttttaccctgaaaacccgcgagggcggggtagcttctgccgatgaacgcgccgatgaagtggtgatcggcgtcggccctgccttcgataaacaccagcatcacactctgatcgatatgccccatggcgcgatcctcaaagagctgattgccggggtggaagaagaggggcttcacgcccgggtggtgcgcattctgcgcacgtccgacgtctcctttatggcctgggatgcggccaacctgagcggctcggggatcggcatcggtatccagtcgaaggggaccacggtcatccatcagcgcgatctgctgccgctcagcaacctggagctgttctcccaggcgccgctgctgacgctggaaacctaccggcagattggcaaaaacgccgcgcgctatgcgcgcaaagagtcaccttcgccggtgccggtggtgaacgatcagatggtgcggccgaaatttatggccaaagccgcgctatttcatatcaaagagaccaaacatgtggtgcaggacgccgagcccgtcaccctgcacgtcgacttagtaagggagtga

SEQ ID NO: 15 - DNA, 426 bp, Klebsiella pneumoniae
  source 1..426: mol_type = genomic DNA
atgagcgagaaaaccatgcgcgtgcaggattatccgttagccacccgctgcccggagcatatcctgacgcctaccggcaaaccattgaccgatattaccctcgagaaggtgctctctggcgaggtgggcccgcaggatgtgcggatctcctgccagacccttgagtaccaggcgcagattgccgagcagatgcagcgccatgcggtggcgcgcaatttccgccgcgcggcggagcttatcgccattcctgacgagcgcattctggctatctataacgcgctgcgcccgttccgctcctcgcaggcggagctgctggcgatcgccgacgagctggagcacacctggcatgcgacagtgaatgccgcctttgtccgggagtcggcggaagtgtatcagcagcggcataagctgcgtaaaggaagctaa

SEQ ID NO: 16 - DNA, 2265 bp, synthetic construct
  source 1..2265: mol_type = other DNA
atgaaaagatcaaaacgatttgcagtactggcccagcgccccgtcaatcaggacgggctgattggcgagtggcctgaagaggggctgatcgccatggacagcccctttgacccggtctcttcagtaaaagtggacaacggtctgatcgtcgagctggacggcaaacgccgggaccagtttgacatgatcgaccgatttatcgccgattacgcgatcaacgttgagcgcacagagcaggcaatgcgcctggaggcggtggaaatagcccgcatgctggtggatattcacgtcagtcgggaggagatcattgccatcactaccgccatcacgccggccaaagcggtcgaggtgatggcgcagatgaacgtggtggagatgatgatggcgctgcagaagatgcgtgcccgccggaccccctccaaccagtgccacgtcaccaatctcaaagataatccggtgcagattgctgctgacgccgccgaggccgggatccgcggcttctcagaacaggagaccacggtcggtatcgcgcgctatgcgccgtttaacgccctggcgctgttggtcggttcgcagtgcggccgccccggcgttttgacgcagtgctcggtggaagaggccaccgagctggagctgggcatgcgtggcttaaccagctacgccgagacggtgtcggtctacggcaccgaagcggtatttaccgacggcgatgatactccgtggtcaaaggcgttcctcgcctcggcctacgcctcccgcgggttgaaaatgcgctacacctccggcaccggatccgaagcgctgatgggctattcggagagcaagtcgatgctctacctcgaatcgcgctgcatcttcattaccaaaggcgccggggttcaggggctgcaaaacggcgcggtgagctgtatcggcatgaccggcgctgtgccgtcgggcattcgggcggtgctggcggaaaacctgatcgcctctatgctcgacctcgaagtggcgtccgccaacgaccagactttctcccactcggatattcgccgcaccgcgcgcaccctgatgcagatgctgccgggcaccgactttattttctccggctacagcgcggtgccgaactacgacaacatgttcgccggctcgaacttcgatgcggaagattttgatgattacaacatcctgcagcgtgacctgatggttgacggcggcctgcgtccggtgaccgaggcggaaaccattgccattcgccagaaagcggcgcgggcgatccaggcggttttccgcgagctggggctgccgccaatcgccgacgaggaggtggaggccgccacctacgcgcacggtagcaacgagatgccgccgcgtaacgtggtggaggatctgagtgcggtggaagagatgatgaagcgcaacatcaccggcctcgatattgtcggcgcgctgagccgcagcggctttgaggatatcgccagcaatattctcaatatgctgcgccagcgggtcaccggcgattacctgcagacctcggccattctcgatcggcagttcgaggtggtgagtgcggtcaacgacatcaatgactatcaggggccgggcaccggctatcgcatctctgccgaacgctgggcggagatcaaaaatattccgggcgtggttcagcccgacaccattgaacaaggcggtattcctgtgcaacagacaacccaaattcagccctcttttaccctgaaaacccgcgagggcggggtagcttctgccgatgaacgcgccgatgaagtggtgatcggcgtcggccctgccttcgataaacaccagcatcacactctgatcgatatgccccatggcgcgatcctcaaagagctgattgccggggtggaagaagaggggcttcacgcccgggtggtgcgcattctgcgcacgtccgacgtctcctttatggcctgggatgcggccaacctgagcggctcggggatcggcatcggtatccagtcgaaggggaccacggtcatccatcagcgcgatctgctgccgctcagcaacctggagctgttctcccaggcgccgctgctgacgctggaaacctaccggcagattggcaaaaacgccgcgcgctatgcgcgcaaagagtcaccttcgccggtgccggtggtgaacgatcagatggtgcggccgaaatttatggccaaagccgcgctatttcatatcaaagagaccaaacatgtggtgcaggacgccgagcccgtcaccctgcacgtcgacttagtaagggagtga

SEQ ID NO: 17 - DNA, 2265 bp, synthetic construct
  source 1..2265: mol_type = other DNA
atgaaaagatcaaaacgatttgcagtactggcccagcgccccgtcaatcaggacgggctgattggcgagtggcctgaagaggggctgatcgccatggacagcccctttgacccggtctcttcagtaaaagtggacaacggtctgatcgtcgagctggacggcaaacgccgggaccagtttgacatgatcgaccgatttatcgccgattacgcgatcaacgttgagcgcacagagcaggcaatgcgcctggaggcggtggaaatagcccgcatgctggtggatattcacgtcagtcgggaggagatcattgccatcactaccgccatcacgccggccaaagcggtcgaggtgatggcgcagatgaacgtggtggagatgatgatggcgctgcagaagatgcgtgcccgccggaccccctccaaccagtgccacgtcaccaatctcaaagataatccggtgcagattgctgctgacgccgccgaggccgggatccgcggcttctcagaacaggagaccacggtcggtatcatgcgctatgcgccgtttaacgccctggcgctgttggtcggttcgcagtgcggccgccccggcgttttgacgcagtgctcggtggaagaggccaccgagctggagctgggcatgcgtggcttaaccagctacgccgagacggtgtcggtctacggcaccgaagcggtatttaccgacggcgatgatactccgtggtcaaaggcgttcctcgcctcggcctacgcctcccgcgggttgaaaatgcgctacacctccggcaccggatccgaagcgctgatgggctattcggagagcaagtcgatgctctacctcgaatcgcgctgcatcttcattaccaaaggcgccggggttcaggggctgcaaaacggcgcggtgagctgtatcggcatgaccggcgctgtgccgtcgggcattcgggcggtgctggcggaaaacctgatcgcctctatgctcgacctcgaagtggcgtccgccaacgaccagactttctcccactcggatattcgccgcaccgcgcgcaccctgatgcagatgctgccgggcaccgactttattttctccggctacagcgcggtgccgaactacgacaacatgttcgccggctcgaacttcgatgcggaagattttgatgattacaacatcctgcagcgtgacctgatggttgacggcggcctgcgtccggtgaccgaggcggaaaccattgccattcgccagaaagcggcgcgggcgatccaggcggttttccgcgagctggggctgccgccaatcgccgacgaggaggtggaggccgccacctacgcgcacggtagcaacgagatgccgccgcgtaacgtggtggaggatctgagtgcggtggaagagatgatgaagcgcaacatcaccggcctcgatattgtcggcgcgctgagccgcagcggctttgaggatatcgccagcaatattctcaatatgctgcgccagcgggtcaccggcgattacctgcagacctcggccattctcgatcggcagttcgaggtggtgagtgcggtcaacgacatcaatgactatcaggggccgggcaccggctatcgcatctctgccgaacgctgggcggagatcaaaaatattccgggcgtggttcagcccgacaccattgaacaaggcggtattcctgtgcaacagacaacccaaattcagccctcttttaccctgaaaacccgcgagggcggggtagcttctgccgatgaacgcgccgatgaagtggtgatcggcgtcggccctgccttcgataaacaccagcatcacactctgatcgatatgccccatggcgcgatcctcaaagagctgattgccggggtggaagaagaggggcttcacgcccgggtggtgcgcattctgcgcacgtccgacgtctcctttatggcctgggatgcggccaacctgagcggctcggggatcggcatcggtatccagtcgaaggggaccacggtcatccatcagcgcgatctgctgccgctcagcaacctggagctgttctcccaggcgccgctgctgacgctggaaacctaccggcagattggcaaaaacgccgcgcgctatgcgcgcaaagagtcaccttcgccggtgccggtggtgaacgatcagatggtgcggccgaaatttatggccaaagccgcgctatttcatatcaaagagaccaaacatgtggtgcaggacgccgagcccgtcaccctgcacgtcgacttagtaagggagtga

SEQ ID NO: 18 - DNA, 2265 bp, synthetic construct
  source 1..2265: mol_type = other DNA
atgaaaagatcaaaacgatttgcagtactggcccagcgccccgtcaatcaggacgggctgattggcgagtggcctgaagaggggctgatcgccatggacagcccctttgacccggtctcttcagtaaaagtggacaacggtctgatcgtcgagctggacggcaaacgccgggaccagtttgacatgatcgaccgatttatcgccgattacgcgatcaacgttgagcgcacagagcaggcaatgcgcctggaggcggtggaaatagcccgcatgctggtggatattcacgtcagtcgggaggagatcattgccatcactaccgccatcacgccggccaaagcggtcgaggtgatggcgcagatgaacgtggtggagatgatgatggcgctgcagaagatgcgtgcccgccggaccccctccaaccagtgccacgtcaccaatctcaaagataatccggtgcagattgctgctgacgccgccgaggccgggatccgcggcttctcagaacaggagaccacggtcggtatcgcgcgctatgcgccgtttaacgccctggcgctgttggtcggttcgcagtgcggccgccccggcgttttgacgcagtgctcggtggaagaggccaccgagctggagctgggcatgcgtggcttaaccagctacgccgagacggtgtcggtctacggcaccgaagcggtatttaccgacggcgatgatactccgtggtcaaaggcgttcctcgcctcggcctacgcctcccgcgggttgaaaatgcgctacacctccggcaccggatccgaagcgctgatgggctattcggagagcaagtcgatgctctacctcgaatcgcgctgcatcttcattaccaaaggcgccggggttcaggggctgcaaaacggcgcggtgagctgtatcggcatgaccggcgctgtgccgtcgggcattcgggcggtgctggcggaaaacctgatcgcctctatgctcgacctcgaagtggcgtccgccaacgaccagactttctcccactcggatattcgccgcaccgcgcgcaccctgatgcagatgctgccgggcaccgactttattttctccggctacagcgcggtgccgaactacgacaacatgttcgccggctcgaacttcgatgcggaagattttgatgattacaacatcctgcagcgtgacctgatggttgacggcggcctgcgtccggtgaccgaggcggaaaccattgccattcgccagaaagcggcgcgggcgatccaggcggttttccgcgagctggggctgccgccaatcgccgacgaggaggtggaggccgccacctacgcgcacggtagcaacgagatgccgccgcgtaacgtgtgggaggatctgagtgcggtggaagagatgatgaagcgcaacatcaccggcctcgatattgtcggcgcgctgagccgcagcggctttgaggatatcgccagcaatattctcaatatgctgcgccagcgggtcaccggcgattacctgcagacctcggccattctcgatcggcagttcgaggtggtgagtgcggtcaacgacatcaatgactatcaggggccgggcaccggctatcgcatctctgccgaacgctgggcggagatcaaaaatattccgggcgtggttcagcccgacaccattgaacaaggcggtattcctgtgcaacagacaacccaaattcagccctcttttaccctgaaaacccgcgagggcggggtagcttctgccgatgaacgcgccgatgaagtggtgatcggcgtcggccctgccttcgataaacaccagcatcacactctgatcgatatgccccatggcgcgatcctcaaagagctgattgccggggtggaagaagaggggcttcacgcccgggtggtgcgcattctgcgcacgtccgacgtctcctttatggcctgggatgcggccaacctgagcggctcggggatcggcatcggtatccagtcgaaggggaccacggtcatccatcagcgcgatctgctgccgctcagcaacctggagctgttctcccaggcgccgctgctgacgctggaaacctaccggcagattggcaaaaacgccgcgcgctatgcgcgcaaagagtcaccttcgccggtgccggtggtgaacgatcagatggtgcggccgaaatttatggccaaagccgcgctatttcatatcaaagagaccaaacatgtggtgcaggacgccgagcccgtcaccctgcacgtcgacttagtaagggagtga

SEQ ID NO: 19 - DNA, 2265 bp, synthetic construct
  source 1..2265: mol_type = other DNA
atgaaaagatcaaaacgatttgcagtactggcccagcgccccgtcaatcaggacgggctgattggcgagtggcctgaagaggggctgatcgccatggacagcccctttgacccggtctcttcagtaaaagtggacaacggtctgatcgtcgagctggacggcaaacgccgggaccagtttgacatgatcgaccgatttatcgccgattacgcgatcaacgttgagcgcacagagcaggcaatgcgcctggaggcggtggaaatagcccgcatgctggtggatattcacgtcagtcgggaggagatcattgccatcactaccgccatcacgccggccaaagcggtcgaggtgatggcgcagatgaacgtggtggagatgatgatggcgctgcagaagatgcgtgcccgccggaccccctccaaccagtgccacgtcaccaatctcaaagataatccggtgcagattgctgctgacgccgccgaggccgggatccgcggcttctcagaacaggagaccacggtcggtatcgcgcgctatgcgccgtttaacgccctggcgctgttggtcggttcgcagtgcggccgccccggcgttttgacgcagtgctcggtggaagaggccaccgagctggagctgggcatgcgtggcttaaccagctacgccgagacggtgtcggtctacggcaccgaagcggtatttaccgacggcgatgatactccgtggtcaaaggcgttcctcgcctcggcctacgcctcccgcgggttgaaaatgcgctacacctccggcaccggatccgaagcgctgatgggctattcggagagcaagtcgatgctctacctcgaatcgcgctgcatcttcattaccaaaggcgccggggttcaggggctgcaaaacggcgcggtgagctgtatcggcatgaccggcgctgtgccgtcgggcattcgggcggtgctggcggaaaacctgatcgcctctatgctcgacctcgaagtggcgtccgccaacgaccagactttctcccactcggatattcgccgcaccgcgcgcaccctgatgcagatgctgccgggcaccgactttattttctccggctacagcgcggtgccgaactacgacaacatgttcgccggctcgaacttcgatgcggaagattttgatgattacaacatcctgcagcgtgacctgatggttgacggcggcctgcgtccggtgaccgaggcggaaaccattgccattcgccagaaagcggcgcgggcgatccaggcggttttccgcgagctggggctgccgccaatcgccgacgaggaggtggaggccgccacctacgcgcacggtagcaacgagatgccgccgcgtaacgtggtggaggatctgagtgcggtggaagagatgatgaagcgcaacatcaccggcctcgatattgtcggcgcgctgagccgcagcggctttgaggatatcgccagcaatattctcaatatgctgcgccagcgggtcaccggcgattacctgcagacctcggccattctcgatcggcagttcgaggtggtgagtgcggtcaacgacatcaatgactatcaggggccgggcaccggctatcgcatctctgccgaacgctgggcggagatcaaaaatattccgggcgtggttcagcccgacaccattgaacaaggcggtattcctgtgcaacagacaacccaaattcagccctcttttaccctgaaaacccgcgagggcggggtagcttctgccgatgaacgcgccgatgaagtggtgatcggcgtcggccctgccttcgataaacaccagcatcacactctgatcgatatgccccatggcgcgatcctcaaagagctgattgccggggtggaagaagaggggcttcacgcccgggtggtgcgcattctgcgcacgtccgacgtctcctttatggcctgggatgcggccaacctgagcggctcggggatcggcatcggtatccagtcgaaggggaccacggtcatccatcagcgcgatctgtggccgctcagcaacctggagctgttctcccaggcgccgctgctgacgctggaaacctaccggcagattggcaaaaacgccgcgcgctatgcgcgcaaagagtcaccttcgccggtgccggtggtgaacgatcagatggtgcggccgaaatttatggccaaagccgcgctatttcatatcaaagagaccaaacatgtggtgcaggacgccgagcccgtcaccctgcacgtcgacttagtaagggagtga

SEQ ID NO: 20 - DNA, 2265 bp, synthetic construct
  source 1..2265: mol_type = other DNA
atgaaaagatcaaaacgatttgcagtactggcccagcgccccgtcaatcaggacgggctgattggcgagtggcctgaagaggggctgatcgccatggacagcccctttgacccggtctcttcagtaaaagtggacaacggtctgatcgtcgagctggacggcaaacgccgggaccagtttgacatgatcgaccgatttatcgccgattacgcgatcaacgttgagcgcacagagcaggcaatgcgcctggaggcggtggaaatagcccgcatgctggtggatattcacgtcagtcgggaggagatcattgccatcactaccgccatcacgccggccaaagcggtcgaggtgatggcgcagatgaacgtggtggagatgatgatggcgctgcagaagatgcgtgcccgccggaccccctccaaccagtgccacgtcaccaatctcaaagataatccggtgcagattgctgctgacgccgccgaggccgggatccgcggcttctcagaacaggagaccacggtcggtatcgcgcgctatgcgccgtttaacgccctggcgctgttggtcggttcgcagtgcggccgccccggcgttttgacgcagtgctcggtggaagaggccaccgagctggagctgggcatgcgtggcttaaccagctacgccgagacggtgtcggtctacggcaccgaagcggtatttaccgacggcgatgatactccgtggtcaaaggcgttcctcgcctcggcctacgcctcccgcgggttgaaaatgcgctacacctccggcaccggatccgaagcgctgatgggctattcggagagcaagtcgatgctctacctcgaatcgcgctgcatcttcattaccaaaggcgccggggttcaggggctgcaaaacggcgcggtgagctgtatcggcatgaccggcgctgtgccgtcgggcattcgggcggtgctggcggaaaacctgatcgcctctatgctcgacctcgaagtggcgtccgccaacgaccagactttctcccactcggatattcgccgcaccgcgcgcaccctgatgcagatgctgccgggcaccgactttattttctccggctacagcgcggtgccgaactacgacaacatgttcgccggctcgaacttcgatgcggaagattttgatgattacaacatcctgcagcgtgacctgatggttgacggcggcctgcgtccggtgaccgaggcggaaaccattgccattcgccagaaagcggcgcgggcgatccaggcggttttccgcgagctggggctgccgccaatcgccgacgaggaggtggaggccgccacctacgcgcacggtagcaacgagatgccgccgcgtaacgtggtggaggatctgagtgcggtggaagagatgatgaagcgcaacatcaccggcctcgatattgtcggcgcgctgagccgcagcggctttgaggatatcgccagcaatattctcaatatgctgcgccagcgggtcaccggcgattacctgcagacctcggccattctcgatcggcagttcgaggtggtgagtgcggtcaacgacatcaatgactatcaggggccgggcaccggctatcgcatctctgccgaacgctgggcggagatcaaaaatattccgggcgtggttcagcccgacaccattgaacaaggcggtattcctgtgcaacagacaacccaaattcagccctcttttaccctgaaaacccgcgagggcggggtagcttctgccgatgaacgcgccgatgaagtggtgatcggcgtcggccctgccttcgataaacaccagcatcacactctgatcgatatgccccatggcgcgatcctcaaagagctgattgccggggtggaagaagaggggcttcacgcccgggtggtgcgcattctgcgcacgtccgacgtctcctttatggcctgggatgcggccaacctgagcggctcggggatcggcatcggtatccagtcgaaggggaccacggtcatccatcagcgcgatctgtttccgctcagcaacctggagctgttctcccaggcgccgctgctgacgctggaaacctaccggcagattggcaaaaacgccgcgcgctatgcgcgcaaagagtcaccttcgccggtgccggtggtgaacgatcagatggtgcggccgaaatttatggccaaagccgcgctatttcatatcaaagagaccaaacatgtggtgcaggacgccgagcccgtcaccctgcacgtcgacttagtaagggagtga

SEQ ID NO: 21 - DNA, 2265 bp, synthetic construct; identical to SEQ ID NO: 18
  source 1..2265: mol_type = other DNA

SEQ ID NO: 22 - DNA, 2265 bp, synthetic construct
  source 1..2265: mol_type = other DNA
atgaaaagatcaaaacgatttgcagtactggcccagcgccccgtcaatcaggacgggctgattggcgagtggcctgaagaggggctgatcgccatggacagcccctttgacccggtctcttcagtaaaagtggacaacggtctgatcgtcgagctggacggcaaacgccgggaccagtttgacatgatcgaccgatttatcgccgattacgcgatcaacgttgagcgcacagagcaggcaatgcgcctggaggcggtggaaatagcccgcatgctggtggatattcacgtcagtcgggaggagatcattgccatcactaccgccatcacgccggccaaagcggtcgaggtgatggcgcagatgaacgtggtggagatgatgatggcgctgcagaagatgcgtgcccgccggaccccctccaaccagtgccacgtcaccaatctcaaagataatccggtgcagattgctgctgacgccgccgaggccgggatccgcggcttctcagaacaggagaccacggtcggtatcatgcgctatgcgccgtttaacgccctggcgctgttggtcggttcgcagtgcggccgccccggcgttttgacgcagtgctcggtggaagaggccaccgagctggagctgggcatgcgtggcttaaccagctacgccgagacggtgtcggtctacggcaccgaagcggtatttaccgacggcgatgatactccgtggtcaaaggcgttcctcgcctcggcctacgcctcccgcgggttgaaaatgcgctacacctccggcaccggatccgaagcgctgatgggctattcggagagcaagtcgatgctctacctcgaatcgcgctgcatcttcattaccaaaggcgccggggttcaggggctgcaaaacggcgcggtgagctgtatcggcatgaccggcgctgtgccgtcgggcattcgggcggtgctggcggaaaacctgatcgcctctatgctcgacctcgaagtggcgtccgccaacgaccagactttctcccactcggatattcgccgcaccgcgcgcaccctgatgcagatgctgccgggcaccgactttattttctccggctacagcgcggtgccgaactacgacaacatgttcgccggctcgaacttcgatgcggaagattttgatgattacaacatcctgcagcgtgacctgatggttgacggcggcctgcgtccggtgaccgaggcggaaaccattgccattcgccagaaagcggcgcgggcgatccaggcggttttccgcgagctggggctgccgccaatcgccgacgaggaggtggaggccgccacctacgcgcacggtagcaacgagatgccgccgcgtaacgtggtggaggatctgagtgcggtggaagagatgatgaagcgcaacatcaccggcctcgatattgtcggcgcgctgagccgcagcggctttgaggatatcgccagcaatattctcaatatgctgcgccagcgggtcaccggcgattacctgcagacctcggccattctcgatcggcagttcgaggtggtgagtgcggtcaacgacatcaatgactatcaggggccgggcaccggctatcgcatctctgccgaacgctgggcggagatcaaaaatattccgggcgtggttcagcccgacaccattgaacaaggcggtattcctgtgcaacagacaacccaaattcagccctcttttaccctgaaaacccgcgagggcggggtagcttctgccgatgaacgcgccgatgaagtggtgatcggcgtcggccctgccttcgataaacaccagcatcacactctgatcgatatgccccatggcgcgatcctcaaagagctgattgccggggtggaagaagaggggcttcacgcccgggtggtgcgcattctgcgcacgtccgacgtctcctttatggcctgggatgcggccaacctgagcggctcggggatcggcatcggtatccagtcgaaggggaccacggtcatccatcagcgcgatctgtggccgctcagcaacctggagctgttctcccaggcgccgctgctgacgctggaaacctaccggcagattggcaaaaacgccgcgcgctatgcgcgcaaagagtcaccttcgccggtgccggtggtgaacgatcagatggtgcggccgaaatttatggccaaagccgcgctatttcatatcaaagagaccaaacatgtggtgcaggacgccgagcccgtcaccctgcacgtcgacttagtaagggagtga

SEQ ID NO: 23 - DNA, 2265 bp, synthetic construct
  source 1..2265: mol_type = other DNA
atgaaaagatcaaaacgatttgcagtactggcccagcgccccgtcaatcaggacgggctgattggcgagtggcctgaagaggggctgatcgccatggacagcccctttgacccggtctcttcagtaaaagtggacaacggtctgatcgtcgagctggacggcaaacgccgggaccagtttgacatgatcgaccgatttatcgccgattacgcgatcaacgttgagcgcacagagcaggcaatgcgcctggaggcggtggaaatagcccgcatgctggtggatattcacgtcagtcgggaggagatcattgccatcactaccgccatcacgccggccaaagcggtcgaggtgatggcgcagatgaacgtggtggagatgatgatggcgctgcagaagatgcgtgcccgccggaccccctccaaccagtgccacgtcaccaatctcaaagataatccggtgcagattgctgctgacgccgccgaggccgggatccgcggcttctcagaacaggagaccacggtcggtatcatgcgctatgcgccgtttaacgccctggcgctgttggtcggttcgcagtgcggccgccccggcgttttgacgcagtgctcggtggaagaggccaccgagctggagctgggcatgcgtggcttaaccagctacgccgagacggtgtcggtctacggcaccgaagcggtatttaccgacggcgatgatactccgtggtcaaaggcgttcctcgcctcggcctacgcctcccgcgggttgaaaatgcgctacacctccggcaccggatccgaagcgctgatgggctattcggagagcaagtcgatgctctacctcgaatcgcgctgcatcttcattaccaaaggcgccggggttcaggggctgcaaaacggcgcggtgagctgtatcggcatgaccggcgctgtgccgtcgggcattcgggcggtgctggcggaaaacctgatcgcctctatgctcgacctcgaagtggcgtccgccaacgaccagactttctcccactcggatattcgccgcaccgcgcgcaccctgatgcagatgctgccgggcaccgactttattttctccggctacagcgcggtgccgaactacgacaacatgttcgccggctcgaacttcgatgcggaagattttgatgattacaacatcctgcagcgtgacctgatggttgacggcggcctgcgtccggtgaccgaggcggaaaccattgccattcgccagaaagcggcgcgggcgatccaggcggttttccgcgagctggggctgccgccaatcgccgacgaggaggtggaggccgccacctacgcgcacggtagcaacgagatgccgccgcgtaacgtggtggaggatctgagtgcggtggaagagatgatgaagcgcaacatcaccggcctcgatattgtcggcgcgctgagccgcagcggctttgaggatatcgccagcaatattctcaatatgctgcgccagcgggtcaccggcgattacctgcagacctcggccattctcgatcggcagttcgaggtggtgagtgcggtcaacgacatcaatgactatcaggggccgggcaccggctatcgcatctctgccgaacgctgggcggagatcaaaaatattccgggcgtggttcagcccgacaccattgaacaaggcggtattcctgtgcaacagacaacccaaattcagccctcttttaccctgaaaacccgcgagggcggggtagcttctgccgatgaacgcgccgatgaagtggtgatcggcgtcggccctgccttcgataaacaccagcatcacactctgatcgatatgccccatggcgcgatcctcaaagagctgattgccggggtggaagaagaggggcttcacgcccgggtggtgcgcattctgcgcacgtccgacgtctcctttatggcctgggatgcggccaacctgagcggctcggggatcggcatcggtatccagtcgaaggggaccacggtcatccatcagcgcgatctgctgccgctcagcaacctggagctgttctcccaggcgccgctgctgacgctggaaacctaccggcagattggcaaaaacgccgcgcgctatgcgcgcaaagagtcaccttcgccggtgccggtggtgaacgatcagtgggtgcggccgaaatttatggccaaagccgcgctatttcatatcaaagagaccaaacatgtggtgcaggacgccgagcccgtcaccctgcacgtcgacttagtaagggagtga

SEQ ID NO: 24 - DNA, 2265 bp, synthetic construct
  source 1..2265: mol_type = other DNA
atgaaaagatcaaaacgatttgcagtactggcccagcgccccgtcaatcaggacgggctgattggcgagtggcctgaagaggggctgatcgccatggacagcccctttgacccggtctcttcagtaaaagtggacaacggtctgatcgtcgagctggacggcaaacgccgggaccagtttgacatgatcgaccgatttatcgccgattacgcgatcaacgttgagcgcacagagcaggcaatgcgcctggaggcggtggaaatagcccgcatgctggtggatattcacgtcagtcgggaggagatcattgccatcactaccgccatcacgccggccaaagcggtcgaggtgatggcgcagatgaacgtggtggagatgatgatggcgctgcagaagatgcgtgcccgccggaccccctccaaccagtgccacgtcaccaatctcaaagataatccggtgcagattgctgctgacgccgccgaggccgggatccgcggcttctcagaacaggagaccacggtcggtatcatgcgctatgcgccgtttaacgccctggcgctgttggtcggttcgcagtgcggccgccccggcgttttgacgcagtgctcggtggaagaggccaccgagctggagctgggcatgcgtggcttaaccagctacgccgagacggtgtcggtctacggcaccgaagcggtatttaccgacggcgatgatactccgtggtcaaaggcgttcctcgcctcggcctacgcctcccgcgggttgaaaatgcgctacacctccggcaccggatccgaagcgctgatgggctattcggagagcaagtcgatgctctacctcgaatcgcgctgcatcttcattaccaaaggcgccggggttcaggggctgcaaaacggcgcggtgagctgtatcggcatgaccggcgctgtgccgtcgggcattcgggcggtgctggcggaaaacctgatcgcctctatgctcgacctcgaagtggcgtccgccaacgaccagactttctcccactcggatattcgccgcaccgcgcgcaccctgatgcagatgctgccgggcaccgactttattttctccggctacagcgcggtgccgaactacgacaacatgttcgccggctcgaacttcgatgcggaagattttgatgattacaacatcctgcagcgtgacctgatggttgacggcggcctgcgtccggtgaccgaggcggaaaccattgccattcgccagaaagcggcgcgggcgatccaggcggttttccgcgagctggggctgccgccaatcgccgacgaggaggtggaggccgccacctacgcgcacggtagcaacgagatgccgccgcgtaacgtggtggaggatctgagtgcggtggaagagatgatgaagcgcaacatcaccggcctcgatattgtcggcgcgctgagccgcagcggctttgaggatatcgccagcaatattctcaatatgctgcgccagcgggtcaccggcgattacctgcagacctcggccattctcgatcggcagttcgaggtggtgagtgcggtcaacgacatcaatgactatcaggggccgggcaccggctatcgcatctctgccgaacgctgggcggagatcaaaaatattccgggcgtggttcagcccgacaccattgaacaaggcggtattcctgtgcaacagacaacccaaattcagccctcttttaccctgaaaacccgcgagggcggggtagcttctgccgatgaacgcgccgatgaagtggtgatcggcgtcggccctgccttcgataaacaccagcatcacactctgatcgatatgccccatggcgcgatcctcaaagagctgattgccggggtggaagaagaggggcttcacgcccgggtggtgcgcattctgcgcacgtccgacgtctcctttatggcctgggatgcggccaacctgagcggctcggggatcggcatcggtatccagtcgaaggggaccacggtcatccatcagcgcgatctgtggccgctcagcaacctggagctgttctcccaggcgccgctgctgacgctggaaacctaccggcagattggcaaaaacgccgcgcgctatgcgcgcaaagagtcaccttcgccggtgccggtggtgaacgatcagtgggtgcggccgaaatttatggccaaagccgcgctatttcatatcaaagagaccaaacatgtggtgcaggacgccgagcccgtcaccctgcacgtcgacttagtaagggagtga